European Patent Application EP 4 389 766 A1, published June 26, 2024. Title: ANTI IGSF1 ANTIBODY AND USE THEREOF. Applicant: Wellmarker Bio Co., LTD. The sequence listing filed with the application follows.

SEQUENCE LISTING (24 sequences)

SEQ ID NO: 1 - protein, 8 aa, Artificial Sequence
  H-CDR1 of WM-A1-3389
GGTFSTYA

SEQ ID NO: 2 - protein, 8 aa, Artificial Sequence
  H-CDR2 of WM-A1-3389
IIPFVGTV

SEQ ID NO: 3 - protein, 11 aa, Artificial Sequence
  H-CDR3 of WM-A1-3389
VRDGGRSYFDS

SEQ ID NO: 4 - protein, 8 aa, Artificial Sequence
  L-CDR1 of WM-A1-3389
TSNIGSNL

SEQ ID NO: 5 - protein, 3 aa, Artificial Sequence
  L-CDR2 of WM-A1-3389
DNH

SEQ ID NO: 6 - protein, 11 aa, Artificial Sequence
  L-CDR3 of WM-A1-3389
VAWDDSLNGYV

SEQ ID NO: 7 - protein, 118 aa, Artificial Sequence
  Variable region of heavy chain of WM-A1-3389
QVQLVQSGAEVKRPGSSVKVSCKASGGTFSTYAISWVRQAPGQGLEWMGRIIPFVGTVDYAQKFQDRVTITADKSTNTAYMELSSLRSEDTAVYYCVRDGGRSYFDSWGPGILVTVSS

SEQ ID NO: 8 - protein, 110 aa, Artificial Sequence
  Variable region of light chain of WM-A1-3389
QFVLTQPPSVSAAPGQDVIISCSGNTSNIGSNLVSWFQQFPETAPKLLIYDNHKRPSGISDRFSGTKSGTSASLAISGLQSEDEADYYCVAWDDSLNGYVFGTGTKVTVL

SEQ ID NO: 9 - DNA, 354 bp, Artificial Sequence
  Polynucleotide coding variable region of heavy chain of WM-A1-3389
caggtgcagctggtacagtctggggctgaggtgaagaggcctgggtcctcggtgaaggtctcctgcaaggcttctggaggcaccttcagcacctatgctatcagctgggtgcgacaggcccctggacaagggcttgagtggatgggaaggatcatccctttcgttggtacagtagactacgcacagaagttccaggacagagtcacaattaccgcggacaaatccacgaacacagcctacatggagctgagcagcctgagatctgaggacacggccgtgtattactgtgtgagagatgggggccgtagttattttgactcctggggcccgggaatcctggtcaccgtctcctca

SEQ ID NO: 10 - DNA, 330 bp, Artificial Sequence
  Polynucleotide coding variable region of light chain of WM-A1-3389
cagttcgtgctgactcagccgccctcagtctctgcggccccagggcaggacgtcatcatctcttgctctggaaacacttccaacattgggagtaaccttgtctcctggttccagcaattcccagagacagcccccaaactcctgatttatgacaatcataagcgaccctcaggaatttctgaccgattctctggcaccaagtctggtacctcagcctccctggccatcagtgggctccagtctgaggatgaggctgattattactgtgtggcatgggatgacagtctgaatggttatgtcttcggaactgggaccaaggtcaccgtccta

SEQ ID NO: 11 - protein, 25 aa, Artificial Sequence
  H-FR1 of WM-A1-3389
QVQLVQSGAEVKRPGSSVKVSCKAS

SEQ ID NO: 12 - protein, 17 aa, Artificial Sequence
  H-FR2 of WM-A1-3389
ISWVRQAPGQGLEWMGR

SEQ ID NO: 13 - protein, 38 aa, Artificial Sequence
  H-FR3 of WM-A1-3389
DYAQKFQDRVTITADKSTNTAYMELSSLRSEDTAVYYC

SEQ ID NO: 14 - protein, 11 aa, Artificial Sequence
  H-FR4 of WM-A1-3389
WGPGILVTVSS

SEQ ID NO: 15 - protein, 25 aa, Artificial Sequence
  L-FR1 of WM-A1-3389
QFVLTQPPSVSAAPGQDVIISCSGN

SEQ ID NO: 16 - protein, 17 aa, Artificial Sequence
  L-FR2 of WM-A1-3389
VSWFQQFPETAPKLLIY

SEQ ID NO: 17 - protein, 36 aa, Artificial Sequence
  L-FR3 of WM-A1-3389
KRPSGISDRFSGTKSGTSASLAISGLQSEDEADYYC

SEQ ID NO: 18 - protein, 10 aa, Artificial Sequence
  L-FR4 of WM-A1-3389
FGTGTKVTVL

SEQ ID NO: 19 - protein, 756 aa, Artificial Sequence
  IGSF1
EETEIVMPTPKPELWAETNFPLAPWKNLTLWCRSPSGSTKEFVLLKDGTGWIATRPASEQVRAAFPLGALTQSHTGSYHCHSWEEMAVSEPSEALELVGTDILPKPVISASPTIRGQELQLRCKGWLAGMGFALYKEGEQEPVQQLGAVGREAFFTIQRMEDKDEGNYSCRTHTEKRPFKWSEPSEPLELVIKEMYPKPFFKTWASPVVTPGARVTFNCSTPHQHMSFILYKDGSEIASSDRSWASPGASAAHFLIISVGIGDGGNYSCRYYDFSIWSEPSDPVELVVTEFYPKPTLLAQPGPVVFPGKSVILRCQGTFQGMRFALLQEGAHVPLQFRSVSGNSADFLLHTVGAEDSGNYSCIYYETTMSNRGSYLSMPLMIWVTDTFPKPWLFAEPSSVVPMGQNVTLWCRGPVHGVGYILHKEGEATSMQLWGSTSNDGAFPITNISGTSMGRYSCCYHPDWTSSIKIQPSNTLELLVTGLLPKPSLLAQPGPMVAPGENMTLQCQGELPDSTFVLLKEGAQEPLEQQRPSGYRADFWMPAVRGEDSGIYSCVYYLDSTPFAASNHSDSLEIWVTDKPPKPSLSAWPSTMFKLGKDITLQCRGPLPGVEFVLEHDGEEAPQQFSEDGDFVINNVEGKGIGNYSCSYRLQAYPDIWSEPSDPLELVGAAGPVAQECTVGNIVRSSLIVVVVVALGVVLAIEWKKWPRLRTRGSETDGRDQTIALEECNQEGEPGTPANSPSSTSQRISVELPVPI

SEQ ID NO: 20 - protein, 784 aa, Artificial Sequence
  IGSF1 with leader sequence and His tag
MGWSYIILFLVATAADVHSQHHHHHHHHEETEIVMPTPKPELWAETNFPLAPWKNLTLWCRSPSGSTKEFVLLKDGTGWIATRPASEQVRAAFPLGALTQSHTGSYHCHSWEEMAVSEPSEALELVGTDILPKPVISASPTIRGQELQLRCKGWLAGMGFALYKEGEQEPVQQLGAVGREAFFTIQRMEDKDEGNYSCRTHTEKRPFKWSEPSEPLELVIKEMYPKPFFKTWASPVVTPGARVTFNCSTPHQHMSFILYKDGSEIASSDRSWASPGASAAHFLIISVGIGDGGNYSCRYYDFSIWSEPSDPVELVVTEFYPKPTLLAQPGPVVFPGKSVILRCQGTFQGMRFALLQEGAHVPLQFRSVSGNSADFLLHTVGAEDSGNYSCIYYETTMSNRGSYLSMPLMIWVTDTFPKPWLFAEPSSVVPMGQNVTLWCRGPVHGVGYILHKEGEATSMQLWGSTSNDGAFPITNISGTSMGRYSCCYHPDWTSSIKIQPSNTLELLVTGLLPKPSLLAQPGPMVAPGENMTLQCQGELPDSTFVLLKEGAQEPLEQQRPSGYRADFWMPAVRGEDSGIYSCVYYLDSTPFAASNHSDSLEIWVTDKPPKPSLSAWPSTMFKLGKDITLQCRGPLPGVEFVLEHDGEEAPQQFSEDGDFVINNVEGKGIGNYSCSYRLQAYPDIWSEPSDPLELVGAAGPVAQECTVGNIVRSSLIVVVVVALGVVLAIEWKKWPRLRTRGSETDGRDQTIALEECNQEGEPGTPANSPSSTSQRISVELPVPI

SEQ ID NO: 21 - protein, 448 aa, Artificial Sequence
  Heavy chain of WM-A1-3389
QVQLVQSGAEVKRPGSSVKVSCKASGGTFSTYAISWVRQAPGQGLEWMGRIIPFVGTVDYAQKFQDRVTITADKSTNTAYMELSSLRSEDTAVYYCVRDGGRSYFDSWGPGILVTVSSASTKGPSVFPLAPSSKSTSGGTAALGCLVKDYFPEPVTVSWNSGALTSGVHTFPAVLQSSGLYSLSSVVTVPSSSLGTQTYICNVNHKPSNTKVDKKVEPKSCDKTHTCPPCPAPELLGGPSVFLFPPKPKDTLMISRTPEVTCVVVDVSHEDPEVKFNWYVDGVEVHNAKTKPREEQYNSTYRVVSVLTVLHQDWLNGKEYKCKVSNKALPAPIEKTISKAKGQPREPQVYTLPPSREEMTKNQVSLTCLVKGFYPSDIAVEWESNGQPENNYKTTPPVLDSDGSFFLYSKLTVDKSRWQQGNVFSCSVMHEALHNHYTQKSLSLSPGK

SEQ ID NO: 22 - protein, 217 aa, Artificial Sequence
  Light chain of WM-A1-3389
QFVLTQPPSVSAAPGQDVIISCSGNTSNIGSNLVSWFQQFPETAPKLLIYDNHKRPSGISDRFSGTKSGTSASLAISGLQSEDEADYYCVAWDDSLNGYVFGTGTKVTVLRTVAAPSVFIFPPSDEQLKSGTASVVCLLNNFYPREAKVQWKVDNALQSGNSQESVTEQDSKDSTYSLSSTLTLSKADYEKHKVYACEVTHQGLSSPVTKSFNRGEC

SEQ ID NO: 23 - DNA, 1344 bp, Artificial Sequence
  Polynucleotide coding heavy chain of WM-A1-3389
caagttcagctggttcagtctggcgccgaagtgaaaagacctggcagcagcgtgaaggtgtcctgcaaagcttctggcggcaccttcagcacctacgccatctcttgggttcgacaggcccctggacaaggcctggaatggatgggcagaatcatcccctttgtgggcaccgtggactacgcccagaaattccaggacagagtgaccatcaccgccgacaagagcaccaacaccgcctacatggaactgagcagcctgagaagcgaggacaccgccgtgtactactgcgtccgagatggcggcagaagctacttcgattcttggggccctggcatcctggtcacagtgtctagcgcctctacaaagggccccagcgttttcccactggctcctagcagcaagagcacaagcggaggaacagccgctctgggctgtctggtcaaggactactttcccgagcctgtgaccgtgtcttggaactctggcgctctgacaagcggcgtgcacacatttccagccgtgctgcaaagcagcggcctgtactctctgagcagcgtcgtgacagtgccaagcagctctctgggcacccagacctacatctgcaatgtgaaccacaagcctagcaacaccaaggtggacaagaaggtggaacccaagtcctgcgacaagacccacacctgtcctccatgtcctgctccagaactgctcggcggaccttccgtgttcctgtttcctccaaagcctaaggacaccctgatgatcagcagaacccctgaagtgacctgcgtggtggtggatgtgtcccacgaggacccagaagtgaagttcaattggtacgtggacggcgtggaagtgcacaacgccaagaccaagcctagagaggaacagtacaactccacctacagagtggtgtccgtgctgacagtgctgcaccaggattggctgaacggcaaagagtacaagtgcaaggtgtccaacaaggccctgcctgctcctatcgagaaaaccatcagcaaggccaagggccagcctagggaaccccaggtttacacactgcctccaagccgggaagagatgacaaagaaccaggtgtccctgacctgcctcgtgaagggcttctacccttccgatatcgccgtggaatgggagagcaatggccagccagagaacaactacaagacaacccctcctgtgctggacagcgacggctcattcttcctgtacagcaagctgaccgtggacaagtccagatggcagcagggcaacgtgttcagctgcagcgtgatgcacgaggccctgcacaaccactacacacagaagtccctgtctctgagccccggcaaa

SEQ ID NO: 24 - DNA, 651 bp, Artificial Sequence
  Polynucleotide coding light chain of WM-A1-3389
cagtttgttctgacacagcctccaagcgtgtccgccgctcctggacaggatgtgatcatcagctgcagcggcaacaccagcaacatcggcagcaatctggtgtcctggttccagcagttccccgagacagcccctaagctgctgatctacgacaaccacaagcggcccagcggcatcagcgatagattcagcggcacaaagagcggcaccagcgcttctctggccatctctggactgcagagcgaggacgaggccgactactattgtgtggcctgggacgacagcctgaacggctatgtgtttggcaccggcaccaaagtgaccgtgctgagaacagtggccgctcctagcgtgttcatcttcccaccttccgacgagcagctgaagtctggcacagccagcgttgtgtgcctgctgaacaacttctaccctcgggaagccaaggtgcagtggaaggtggacaatgccctgcagtccggcaacagccaagagagcgtgacagagcaggacagcaaggactccacctacagcctgagcagcaccctgacactgagcaaggccgattacgagaagcacaaggtgtacgcctgcgaagtgacacaccagggcctgtctagccctgtgaccaagagcttcaacagaggcgagtgc